European Patent Specification EP 3 775 894 B1, published April 24, 2024. Title: Method for predicting human immune response. Applicant: OBI Pharma Inc. The sequence listing filed with the application follows.

SEQUENCE LISTING (1 sequence)

SEQ ID NO: 1 - DNA, 696 bp, Artificial Sequence
  fluorescent protein
atggcccagtccaagcacggcctgaccaaggagatgaccatgaagtaccgcatggagggctgcgtggacggccacaagttcgtgatcaccggcgagggcatcggctaccccttcaagggcaagcaggccatcaacctgtgcgtggtggagggcggccccttgcccttcgccgaggacatcttgtccgccgccttcatgtacggcaaccgcgtgttcaccgagtacccccaggacatcgtcgactacttcaagaactcctgccccgccggctacacctgggaccgctccttcctgttcgaggacggcgccgtgtgcatctgcaacgccgacatcaccgtgagcgtggaggagaactgcatgtaccacgagtccaagttctacggcgtgaacttccccgccgacggccccgtgatgaagaagatgaccgacaactgggagccctcctgcgagaagatcatccccgtgcccaagcagggcatcttgaagggcgacgtgagcatgtacctgctgctgaaggacggtggccgcttgcgctgccagttcgacaccgtgtacaaggccaagtccgtgccccgcaagatgcccgactggcacttcatccagcacaagctgacccgcgaggaccgcagcgacgccaagaaccagaagtggcacctgaccgagcacgccatcgcctccggctccgccttgccctga